European Patent Application EP 4 667 579 A1, published December 24, 2025. Title: MICROORGANISMS FOR PRODUCING PHB AND PROCESS FOR PRODUCING PHB USING THE SAME. Applicant: 씨제이제일제당 (주). The sequence listing filed with the application follows.

SEQUENCE LISTING (12 sequences)

SEQ ID NO: 1 - protein, 389 aa, Methylosinus sp.
MDVHEYQAKELLASCGVAVPPGTVAFSPDQAVYAATELGGSHWVVKAQIHAGARGKAGGVKLCRTYHEVQQAARELLGKRLVTKQTGPEGKPVQRVYVELADPYERELYLGFVLDRKLERVRVIASKHGGMEIEEIAKTDPDAILQVIVEPAVGLLPFQARELAFQLGLNLKQVSRAVQSILGAYRAFRDNDATMLEINPLVVTKDDKVLALDAKMSFDDNALFRRRNIVDMNDPSQSDPREAQALEHSLNYIGLDGEIGCIVNGAGLAMATMDMIKHAGGNPANFLDVGGGASAERVATAFRLVLSDANVKVVLVNIFAGINRCDWVAQGVVDAVKATNITAPLVVRLAGTNVEAGRKLLDESGINVITADSLADAAQKAVAAWRSVK

SEQ ID NO: 2 - protein, 295 aa, Methylosinus sp.
MSILIDEKTPILVQGITGDKGSFHAKEMIDYGTNVVAGVTPGKGGKTVHGVPIFDTVREAVKQTGATTSITFVAPPFAADAIMEAADAGIHLICSITDGIPAQDMMRVKRYFLRYPRERRPMMVGPNCAGIISPGKAMLGIMPGHIYKQGNVGLISRSGTLGYEAASQLKELGLGISTSVGIGGDPINGSSFLDHLVLFDQDPETEAVLIIGEIGGPQEAEAAAWIKENFSKPVVGFVAGLTAPKGRRMGHAGAIISATGDSAAEKTEIMKSYGLAVAPSPAEFGSAVAAVLKRA

SEQ ID NO: 3 - DNA, 1170 bp, Methylosinus sp.
  source 1..1170: mol_type = genomic DNA
atggacgtccatgagtatcaagccaaagaattattggcgagctgcggcgtcgcggtgccccccggcaccgtcgctttcagccccgatcaggccgtttacgcggcgaccgagctcggcggctcgcattgggtggtgaaggcgcagattcatgccggcgcgcgcggcaaggcgggcggcgtcaagctgtgccgcacctatcacgaggttcagcaggccgcgcgcgaattgctcggcaagcgtctcgtcaccaagcagaccgggccggaaggcaagccggtgcagcgcgtctatgtcgaactcgccgacccctatgagcgcgagctctatctcggcttcgtcctcgaccgcaagctcgagcgcgtgcgcgtcatcgcctccaagcatggcggcatggagatcgaggagatcgccaagaccgatcccgacgccattctccaggtcatcgtcgagccggccgtcggcctgctgcccttccaggcgcgcgagctggcctttcagctcggcctcaatctcaagcaggtgtcgcgcgcggttcagtcgatcctcggcgcctatcgcgccttccgcgacaatgacgcgaccatgctggagatcaatccgctggtcgtcaccaaggacgacaaggttctcgcgctcgacgcgaaaatgtccttcgacgacaacgctctcttccgtcgccgcaacatcgtcgacatgaacgatccctcgcagtccgacccgcgcgaggcgcaggcgctcgagcattcgctcaactacatcggcctcgacggcgagatcggctgcatcgtcaatggcgcgggcctcgcgatggcgacgatggacatgatcaagcacgccggcggcaatccggcgaacttcctcgacgtcggcggcggcgcctcggccgagcgcgtcgcgacggcgttccgtctcgtgctctccgacgccaatgtgaaggtggtgctcgtcaacatcttcgccggcatcaatcgctgcgactgggtcgcgcaaggcgtcgtcgacgcggtgaaggcgaccaacatcactgcgccgctcgtcgtgcgtctcgccggcaccaatgtcgaggccggccgcaagctgctcgacgagagcggcatcaatgtcatcaccgccgattcgctggccgacgccgcccaaaaggccgtcgccgcttggcgctccgtgaagtga

SEQ ID NO: 4 - DNA, 888 bp, Methylosinus sp.
  source 1..888: mol_type = genomic DNA
atgagcattctcatcgacgaaaaaacgcccatcctcgtccagggcatcaccggcgacaagggcagctttcacgccaaggagatgatcgactacggcacgaatgtcgtcgccggcgtcactccgggcaaaggcgggaagaccgtgcatggcgtgccgatcttcgacacggtgcgcgaggcggtgaagcagaccggcgcgaccaccagcatcactttcgtggccccgccattcgcggccgacgcgatcatggaggcggcggacgccggcattcatctcatctgctccatcaccgatggcattccggctcaggacatgatgcgcgtgaagcgctatttcctgcgctatccgcgcgagcgccggccgatgatggtcgggccgaactgcgccggcatcatcagccccggcaaggccatgctcggcatcatgcccggccacatctacaagcagggcaacgtcggcctcatctcgcgctccggcacgctcggctatgaggcggcctcgcagctgaaggaactcgggctcggcatctcgacctcggtcggcatcggcggcgatcccatcaacggctcgtccttcctcgatcatctcgtgctgttcgatcaggacccggagacggaagcagttctgatcatcggcgagatcggcggtccgcaggaggccgaggccgcggcctggatcaaggagaatttctccaagccggtggtcggcttcgtcgccggcctcaccgcgcccaagggccgccgcatgggccatgcgggcgccatcatctcggcgaccggcgacagcgccgcggagaagaccgagatcatgaagtcctacggcctcgccgtggcgccgagcccggccgagttcggctccgccgtcgccgccgtgctgaagcgcgcgtga

SEQ ID NO: 5 - DNA, 22 bp, unidentified
  source 1..22: mol_type = genomic DNA
gcggcgaggccgggaggaaaca

SEQ ID NO: 6 - DNA, 2080 bp, synthetic construct
  source 1..2080: mol_type = other DNA
atggacgtccatgagtatcaagccaaagaattattggcgagctgcggcgtcgcggtgccccccggcaccgtcgctttcagccccgatcaggccgtttacgcggcgaccgagctcggcggctcgcattgggtggtgaaggcgcagattcatgccggcgcgcgcggcaaggcgggcggcgtcaagctgtgccgcacctatcacgaggttcagcaggccgcgcgcgaattgctcggcaagcgtctcgtcaccaagcagaccgggccggaaggcaagccggtgcagcgcgtctatgtcgaactcgccgacccctatgagcgcgagctctatctcggcttcgtcctcgaccgcaagctcgagcgcgtgcgcgtcatcgcctccaagcatggcggcatggagatcgaggagatcgccaagaccgatcccgacgccattctccaggtcatcgtcgagccggccgtcggcctgctgcccttccaggcgcgcgagctggcctttcagctcggcctcaatctcaagcaggtgtcgcgcgcggttcagtcgatcctcggcgcctatcgcgccttccgcgacaatgacgcgaccatgctggagatcaatccgctggtcgtcaccaaggacgacaaggttctcgcgctcgacgcgaaaatgtccttcgacgacaacgctctcttccgtcgccgcaacatcgtcgacatgaacgatccctcgcagtccgacccgcgcgaggcgcaggcgctcgagcattcgctcaactacatcggcctcgacggcgagatcggctgcatcgtcaatggcgcgggcctcgcgatggcgacgatggacatgatcaagcacgccggcggcaatccggcgaacttcctcgacgtcggcggcggcgcctcggccgagcgcgtcgcgacggcgttccgtctcgtgctctccgacgccaatgtgaaggtggtgctcgtcaacatcttcgccggcatcaatcgctgcgactgggtcgcgcaaggcgtcgtcgacgcggtgaaggcgaccaacatcactgcgccgctcgtcgtgcgtctcgccggcaccaatgtcgaggccggccgcaagctgctcgacgagagcggcatcaatgtcatcaccgccgattcgctggccgacgccgcccaaaaggccgtcgccgcttggcgctccgtgaagtgagcggcgaggccgggaggaaacaatgagcattctcatcgacgaaaaaacgcccatcctcgtccagggcatcaccggcgacaagggcagctttcacgccaaggagatgatcgactacggcacgaatgtcgtcgccggcgtcactccgggcaaaggcgggaagaccgtgcatggcgtgccgatcttcgacacggtgcgcgaggcggtgaagcagaccggcgcgaccaccagcatcactttcgtggccccgccattcgcggccgacgcgatcatggaggcggcggacgccggcattcatctcatctgctccatcaccgatggcattccggctcaggacatgatgcgcgtgaagcgctatttcctgcgctatccgcgcgagcgccggccgatgatggtcgggccgaactgcgccggcatcatcagccccggcaaggccatgctcggcatcatgcccggccacatctacaagcagggcaacgtcggcctcatctcgcgctccggcacgctcggctatgaggcggcctcgcagctgaaggaactcgggctcggcatctcgacctcggtcggcatcggcggcgatcccatcaacggctcgtccttcctcgatcatctcgtgctgttcgatcaggacccggagacggaagcagttctgatcatcggcgagatcggcggtccgcaggaggccgaggccgcggcctggatcaaggagaatttctccaagccggtggtcggcttcgtcgccggcctcaccgcgcccaagggccgccgcatgggccatgcgggcgccatcatctcggcgaccggcgacagcgccgcggagaagaccgagatcatgaagtcctacggcctcgccgtggcgccgagcccggccgagttcggctccgccgtcgccgccgtgctgaagcgcgcgtga

SEQ ID NO: 7 - DNA, 44 bp, synthetic construct
  source 1..44: mol_type = other DNA
cgtcaaaagggcgacaccccctaattagcccgggcgaaaggccc

SEQ ID NO: 8 - DNA, 55 bp, synthetic construct
  source 1..55: mol_type = other DNA
cgcccctacggcgcccactgctctagaggatcccctttgcctggcggcagtagcg

SEQ ID NO: 9 - DNA, 41 bp, synthetic construct
  source 1..41: mol_type = other DNA
ttcacacaggaaacagctatggacgtccatgagtatcaagc

SEQ ID NO: 10 - DNA, 39 bp, synthetic construct
  source 1..39: mol_type = other DNA
ggggtgtcgcccttttgacgtcacgcgcgcttcagcacg

SEQ ID NO: 11 - DNA, 39 bp, synthetic construct
  source 1..39: mol_type = other DNA
cagtgggcgccgtaggggcggcgtaatgctctgccagtg

SEQ ID NO: 12 - DNA, 24 bp, synthetic construct
  source 1..24: mol_type = other DNA
catagctgtttcctgtgtgaatac